European Patent Specification EP 3 452 096 B1, published January 29, 2025. Title: BICYCLIC PEPTIDE-TOXIN CONJUGATES SPECIFIC FOR MT1-MMP. Applicant: BICYCLE THERAPEUTICS LIMITED. The sequence listing filed with the application follows.

SEQUENCE LISTING (15 sequences)

SEQ ID NO: 1 - protein, 14 aa, Artificial
  Synthetic Peptide
  misc_feature (2)..(5): Xaa can be any naturally occurring amino acid
  misc_feature (12)..(13): Xaa can be any naturally occurring amino acid
CXXXXGCEDFYXXC

SEQ ID NO: 2 - protein, 14 aa, Artificial
  Synthetic Peptide
CYNEFGCEDFYDIC

SEQ ID NO: 3 - protein, 15 aa, Artificial
  Synthetic Peptide
ACYNEFGCEDFYDIC

SEQ ID NO: 4 - protein, 15 aa, Artificial
  Synthetic Peptide
CDANEFGCEDFYDIC

SEQ ID NO: 5 - protein, 17 aa, Artificial
  Synthetic Peptide
  misc_feature (2)..(2): Xaa can be any naturally occurring amino acid
  misc_feature (8)..(8): Xaa can be any naturally occurring amino acid
  misc_feature (16)..(16): Xaa can be any naturally occurring amino acid
AXACANEXACEDFYDXC

SEQ ID NO: 6 - protein, 14 aa, Artificial
  Synthetic Peptide
  misc_feature (2)..(5): Xaa can be any naturally occurring amino acid
  misc_feature (12)..(13): Xaa can be any naturally occurring amino acid
CXXXXGCEDFYXXC

SEQ ID NO: 7 - protein, 14 aa, Artificial
  Synthetic Peptide
  misc_feature (2)..(4): Xaa can be any naturally occurring amino acid
CXXXFGCEDFYDIC

SEQ ID NO: 8 - protein, 14 aa, Artificial
  Synthetic Peptide
  misc_feature (2)..(4): Xaa can be any naturally occurring amino acid
CXXXFGCEDFYDIC

SEQ ID NO: 9 - protein, 14 aa, Artificial
  Synthetic Peptide
  misc_feature (2)..(2): Xaa can be any naturally occurring amino acid
  misc_feature (4)..(4): Xaa can be any naturally occurring amino acid
CXNXFGCEDFYDIC

SEQ ID NO: 10 - protein, 14 aa, Artificial
  Synthetic Peptide
CMNQFGCEDFYDIC

SEQ ID NO: 11 - protein, 14 aa, Artificial
  Synthetic Peptide
CFGEFGCEDFYDIC

SEQ ID NO: 12 - protein, 14 aa, Artificial
  Synthetic Peptide
CVNEFGCEDFYDIC

SEQ ID NO: 13 - protein, 14 aa, Artificial
  Synthetic Peptide
CFNEFGCEDFYDIC

SEQ ID NO: 14 - protein, 14 aa, Artificial
  Synthetic Peptide
CYNEYGCEDFYDIC

SEQ ID NO: 15 - protein, 14 aa, Artificial
  Synthetic Peptide
CYNEWGCEDFYDIC